European Patent Specification EP 3 981 435 B1, published August 16, 2023. Title: Lipid composition. Applicant: FUJIFILM Corporation. The sequence listing filed with the application follows.

SEQUENCE LISTING (2 sequences)

SEQ ID NO: 1 - RNA, 21 nt, Artificial Sequence
  Description of Artificial Sequence: siRNA
ggacaggccuguacaacuatt

SEQ ID NO: 2 - RNA, 21 nt, Artificial Sequence
  Description of Artificial Sequence: siRNA
ttccuguccggacauguugau